European Patent Specification EP 3 789 380 B1, published December 4, 2024. Title: Novel ASM direct inhibition compound 2-amino-2-(1,2,3-triazol-4-yl)propane-1,3-diol derivatives and uses thereof. Applicant: Kyungpook National University Industry-Academic Cooperation Foundation. The sequence listing filed with the application follows.

SEQUENCE LISTING (8 sequences)

SEQ ID NO: 1 - DNA, 20 bp, Artificial Sequence
  mTNF-a forward
gattatggctcagggtccaa

SEQ ID NO: 2 - DNA, 20 bp, Artificial Sequence
  mTNF-a reverse
gctccagtgaattcggaaag

SEQ ID NO: 3 - DNA, 20 bp, Artificial Sequence
  mIL-1b forward
cccaagcaatacccaaagaa

SEQ ID NO: 4 - DNA, 20 bp, Artificial Sequence
  mIL-1b reverse
gcttgtgctctgcttgtgag

SEQ ID NO: 5 - DNA, 20 bp, Artificial Sequence
  mIL-6 forward
ccggagaggagacttcacag

SEQ ID NO: 6 - DNA, 20 bp, Artificial Sequence
  mIL-6 reverse
ttgccattgcacaactcttt

SEQ ID NO: 7 - DNA, 20 bp, Artificial Sequence
  mGAPDH forward
tgaatacggctacagcaaca

SEQ ID NO: 8 - DNA, 20 bp, Artificial Sequence
  mGAPDH reverse
aggcccctcctgttattatg